European Patent Application EP 4 357 359 A1, published April 24, 2024. Title: G-PROTEIN-GATED-K+ CHANNEL-MEDIATED ENHANCEMENTS IN LIGHT SENSITIVITY IN ROD-CONE DYSTROPHY (RCD). Applicant: SPARINGVISION. Application EP. The sequence listing filed with the application follows.

SEQUENCE LISTING (21 sequences)

SEQ ID NO: 1 - protein, 419 aa, Homo sapiens
MAGDSRNAMNQDMEIGVTPWDPKKIPKQARDYVPIATDRTRLLAEGKKPRQRYMEKSGKCNVHHGNVQETYRYLSDLFTTLVDLKWRFNLLVFTMVYTVTWLFFGFIWWLIAYIRGDLDHVGDQEWIPCVENLSGFVSAFLFSIETETTIGYGFRVITEKCPEGIILLLVQAILGSIVNAFMVGCMFVKISQPKKRAETLMFSNNAVISMRDEKLCLMFRVGDLRNSHIVEASIRAKLIKSRQTKEGEFIPLNQTDINVGFDTGDDRLFLVSPLIISHEINQKSPFWEMSQAQLHQEEFEVVVILEGMVEATGMTCQARSSYMDTEVLWGHRFTPVLTLEKGFYEVDYNTFHDTYETNTPSCCAKELAEMKREGRLLQYLPSPPLLGGCAEAGLDAEAEQNEEDEPKGLGGSREARGSV

SEQ ID NO: 2 - protein, 419 aa, synthetic construct
MAGDSRNAMNQDMEIGVTPWDPKKIPKQARDYVPIATDRTRLLAEGKKPRQRYMEKSGKCNVHHGNVQETYRYLSDLFTTLVDLKWRFNLLVFTMVYTVTWLFFGFIWWLIAYIRGDLDHVGDQEWIPCVENLSGFVSAFLFTIETETTIGYGFRVITEKCPEGIILLLVQAILGSIVNAFMVGCMFVKISQPKKRAETLMFSNNAVISMRDEKLCLMFRVGDLRNSHIVEASIRAKLIKSRQTKEGEFIPLNQTDINVGFDTGDDRLFLVSPLIISHEINQKSPFWEMSQAQLHQEEFEVVVILEGMVEATGMTCQARSSYMDTEVLWGHRFTPVLTLEKGFYEVDYNTFHDTYETNTPSCCAKELAEMKREGRLLQYLPSPPLLGGCAEAGLDAEAEQNEEDEPKGLGGSREARGSV

SEQ ID NO: 3 - DNA, 1257 bp, synthetic construct
  source 1..1257: mol_type = other DNA
atggccggcgatagcagaaacgccatgaaccaggacatggaaatcggcgtgaccccttgggaccccaagaagattcctaagcaggcccgggactacgtgccaatcgccaccgatagaacaagactgctggccgagggcaagaagcccagacagcggtacatggaaaagtccggcaagtgcaacgtgcaccacggcaatgtgcaagagacatacagatacctgagcgacctgttcaccacactggtggacctgaagtggcggttcaacctgctggtgtttaccatggtgtacacagtgacctggctgttcttcggcttcatctggtggctgatcgcctacatcagaggcgacctggatcacgtgggcgaccaagagtggatcccctgcgtggaaaatctgagcggcttcgtgtccgccttcctgttcacaatcgagacagagacaaccatcggctacggcttcagagtgatcaccgagaagtgccccgagggcatcattctgctgctggtgcaagccatcctgggcagcatcgtgaacgccttcatggtcggatgcatgttcgtgaagatcagccagcctaagaagcgggccgagacactgatgttcagcaacaacgccgtgatcagcatgcgggacgagaagctgtgcctgatgtttagagtgggcgatctgcggaacagccacatcgtggaagccagcatcagagccaagctgatcaagagccggcagaccaaagagggcgagttcatccctctgaaccagaccgacatcaacgtgggcttcgacaccggcgacgacagactgtttctggtgtcccctctgatcatctcccacgagatcaaccagaagtccccattctgggagatgtctcaggcccagctgcaccaagaggaattcgaggtggtggtcatcctggaaggcatggtggaagctaccggcatgacctgtcaggccagatccagctacatggacaccgaggtgctgtggggccacagattcacacctgtgctgaccctggaaaagggcttctacgaggtggactacaacaccttccacgacacctacgagacaaacacccctagctgctgcgccaaagaactggccgagatgaagagagagggcagactgctgcagtacctgccttctccacctctgcttggaggatgtgccgaagccggactggatgccgaggccgaacagaacgaggaagatgagcctaaaggcctcggcggcagcagagaagctagaggatctgtt

SEQ ID NO: 4 - DNA, 234 bp, synthetic construct
  source 1..234: mol_type = other DNA
ccagcaaatccctctgagccgcccccgggggctcgcctcaggagcaaggaagcaaggggtgggaggaggaggtctaagtcccaggcccaattaagagatcagatggtgtaggatttgggagcttttaaggtgaagaggcccgggctgatcccactggccggtataaagcaccgtgaccctcaggtgacgcaccagggccggctgccgtcggggacagggctttccatagcccag

SEQ ID NO: 5 - DNA, 1958 bp, synthetic construct
  source 1..1958: mol_type = other DNA
cctacagcagccagggtgagattatgaggctgagctgagaatatcaagactgtaccgagtagggggccttggcaagtgtggagagcccggcagctggggcagagggcggagtacggtgtgcgtttacggacctcttcaaacgaggtaggaaggtcagaagtcaaaaagggaacaaatgatgtttaaccacacaaaaatgaaaatccaatggttggatatccattccaaatacacaaaggcaacggataagtgatccgggccaggcacagaaggccatgcacccgtaggattgcactcagagctcccaaatgcataggaatagaagggtgggtgcaggaggctgaggggtggggaaagggcatgggtgtttcatgaggacagagcttccgtttcatgcaatgaaaagagtttggagacggatggtggtgactggactatacacttacacacggtagcgatggtacactttgtattatgtatattttaccacgatctttttaaagtgtcaaaggcaaatggccaaatggttccttgtcctatagctgtagcagccatcggctgttagtgacaaagcccctgagtcaagatgacagcagcccccataactcctaatcggctctcccgcgtggagtcatttaggagtagtcgcattagagacaagtccaacatctaatcttccaccctggccagggccccagctggcagcgagggtgggagactccgggcagagcagagggcgctgacattggggcccggcctggcttgggtccctctggcctttccccaggggccctctttccttggggctttcttgggccgccactgctcccgctcctctccccccatcccaccccctcaccccctcgttcttcatatccttctctagtgctccctccactttcatccacccttctgcaagagtgtgggaccacaaatgagttttcacctggcctggggacacacgtgcccccacaggtgctgagtgactttctaggacagtaatctgctttaggctaaaatgggacttgatcttctgttagccctaatcatcaattagcagagccggtgaaggtgcagaacctaccgcctttccaggcctcctcccacctctgccacctccactctccttcctgggatgtgggggctggcacacgtgtggcccagggcattggtgggattgcactgagctgggtcattagcgtaatcctggacaagggcagacagggcgagcggagggccagctccggggctcaggcaaggctgggggcttcccccagacaccccactcctcctctgctggacccccacttcatagggcacttcgtgttctcaaagggcttccaaatagcatggtggccttggatgcccagggaagcctcagagttgcttatctccctctagacagaaggggaatctcggtcaagagggagaggtcgccctgttcaaggccacccagccagctcatggcggtaatgggacaaggctggccagccatcccaccctcagaagggacccggtggggcaggtgatctcagaggaggctcacttctgggtctcacattcttccagcaaatccctctgagccgcccccgggggctcgcctcaggagcaaggaagcaaggggtgggaggaggaggtctaagtcccaggcccaattaagagatcagatggtgtaggatttgggagcttttaaggtgaagaggcccgggctgatcccactggccggtataaagcaccgtgaccctcaggtgacgcaccagggccggctgccgtcggggacagggctttccatagcccaggtaagtatcaaggttacaagacaggtttaaggagaccaatagaaactgggcttgtcgagacagagaagactcttgcgtttctgataggcacctattggtcttactgacatccactttgcctttctctccacaggcccagagaggagacaggccgccacc

SEQ ID NO: 6 - protein, 410 aa, Homo sapiens
MVLKAEHTRSPSATLPSNVPSCRSLSSSEDGPSGPSSLADGGLAHNLQDSVRHRILYLSEQLRVEKASRDGNTVSYLKLVSKADRHQVPHIQQAFEKVNQRASATIAQIEHRLHQCHQQLQELEEGCRPEGLLLMAESDPANCEPPSEKALLSEPPEPGGEDGPVNLPHASRPFILESRFQSLQQGTCLETEDVAQQQNLLLQKVKAELEEAKRFHISLQESYHSLKERSLTDLQLLLESLQEEKCRQALMEEQVNGRLQGQLNEIYNLKHNLACSEERMAYLSYERAKEIWEITETFKSRISKLEMLQQVTQLEAAEHLQSRPPQMLFKFLSPRLSLATVLLVFVSTLCACPSSLISSRLCTCTMLMLIGLGVLAWQRWRAIPATDWQEWVPSRCRLYSKDSGPPADGP

SEQ ID NO: 7 - protein, 7 aa, synthetic construct
LGETTRP

SEQ ID NO: 8 - protein, 732 aa, Adeno-associated virus 9
MAADGYLPDWLEDNLSEGIREWWALKPGAPQPKANQQHQDNARGLVLPGYKYLGPGNGLDKGEPVNAADAAALEHDKAYDQQLKAGDNPYLKYNHADAEFQERLKEDTSFGGNLGRAVFQAKKRLLEPLGLVEEAAKTAPGKKRPVEQSPQEPDSSAGIGKSGAQPAKKRLNFGQTGDTESVPDPQPIGEPPAAPSGVGSLTMASGGGAPVADNNEGADGVGSSSGNWHCDSQWLGDRVITTSTRTWALPTYNNHLYKQISNSTSGGSSNDNAYGYSTPWGYFDFNRFHCHFSPRDWQRLINNNWGFRPKRLNFKLFNIQVKEVTDNNGVKTIANNLTSTVQVFTDSDYQLPYVLGSAHEGCLPPFPADVFMIPQYGYLTLNDGSQAVGRSSFYCLEYFPSQMLRTGNNFQFSYEFENVPFHSSYAHSQSLDRLMNPLIDQYLYYLSKTINGSGQNQQTLKFSVAGPSNMAVQGRNYIPGPSYRQQRVSTTVTQNNNSEFAWPGASSWALNGRNSLMNPGPAMASHKEGEDRFFPLSGSLIFGKQGTGRDNVDADKVMITNEEEIKTTNPVATESYGQVATNHQSAQQAQTGWVQNQGILPGMVWQDRDVYLQGPIWAKIPHTDGNFHPSPLMGGFGMKHPPPQILIKNTPVPADPPTAFNKDKLNSFITQYSTGQVSVEIEWELQKENSKRWNPEIQYTSNYYKSNNVEFAVNTEGVYSEPRPIGTRYLTR

SEQ ID NO: 9 - protein, 735 aa, Adeno-associated virus 2 [sequence omitted]

SEQ ID NO: 10 - protein, 10 aa, synthetic construct
AALGETTRPA

SEQ ID NO: 11 - protein, 10 aa, synthetic construct
LALGETTRPA

SEQ ID NO: 12 - protein, 9 aa, synthetic construct
GLGETTRPA

SEQ ID NO: 13 - DNA, 1724 bp, synthetic construct
  source 1..1724: mol_type = other DNA
ggaggctgaggggtggggaaagggcatgggtgtttcatgaggacagagcttccgtttcatgcaatgaaaagagtttggagacggatggtggtgactggactatacacttacacacggtagcgatggtacactttgtattatgtatattttaccacgatctttttaaagtgtcaaaggcaaatggccaaatggttccttgtcctatagctgtagcagccatcggctgttagtgacaaagcccctgagtcaagatgacagcagcccccataactcctaatcggctctcccgcgtggagtcatttaggagtagtcgcattagagacaagtccaacatctaatcttccaccctggccagggccccagctggcagcgagggtgggagactccgggcagagcagagggcgctgacattggggcccggcctggcttgggtccctctggcctttccccaggggccctctttccttggggctttcttgggccgccactgctcccgctcctctccccccatcccaccccctcaccccctcgttcttcatatccttctctagtgctccctccactttcatccacccttctgcaagagtgtgggaccacaaatgagttttcacctggcctggggacacacgtgcccccacaggtgctgagtgactttctaggacagtaatctgctttaggctaaaatgggacttgatcttctgttagccctaatcatcaattagcagagccggtgaaggtgcagaacctaccgcctttccaggcctcctcccacctctgccacctccactctccttcctgggatgtgggggctggcacacgtgtggcccagggcattggtgggattgcactgagctgggtcattagcgtaatcctggacaagggcagacagggcgagcggagggccagctccggggctcaggcaaggctgggggcttcccccagacaccccactcctcctctgctggacccccacttcatagggcacttcgtgttctcaaagggcttccaaatagcatggtggccttggatgcccagggaagcctcagagttgcttatctccctctagacagaaggggaatctcggtcaagagggagaggtcgccctgttcaaggccacccagccagctcatggcggtaatgggacaaggctggccagccatcccaccctcagaagggacccggtggggcaggtgatctcagaggaggctcacttctgggtctcacattcttggatccggttccaggcctcggccctaaatagtctccctgggctttcaagagaaccacatgagaaaggaggattcgggctctgagcagtttcaccacccaccccccagtctgcaaatcctgacccgtgggtccacctgccccaaaggcggacgcaggacagtagaagggaacagagaacacataaacacagagagggccacagcggctcccacagtcaccgccaccttcctggcggggatgggtggggcgtctgagtttggttcccagcaaatccctctgagccgcccttgcgggctcgcctcaggagcaggggagcaagaggtgggaggaggaggtctaagtcccaggcccaattaagagatcaggtagtgtagggtttgggagcttttaaggtgaagaggcccgggctgatcccacaggccagtataaagcgccgtgaccctcaggtgatgcgccagggccggctgccgtcggggacagggctttccatagcc

SEQ ID NO: 14 - protein, 7 aa, synthetic construct
NETITRP

SEQ ID NO: 15 - protein, 7 aa, synthetic construct
KAGQANN

SEQ ID NO: 16 - protein, 7 aa, synthetic construct
KDPKTTN

SEQ ID NO: 17 - protein, 7 aa, synthetic construct
KDTDTTR

SEQ ID NO: 18 - protein, 7 aa, synthetic construct
RAGGSVG

SEQ ID NO: 19 - protein, 7 aa, synthetic construct
AVDTTKF

SEQ ID NO: 20 - protein, 7 aa, synthetic construct
STGKVPN

SEQ ID NO: 21 - protein, 10 aa, synthetic construct
LAISDQTKHA